European Patent Application EP 4 793 641 A1, published August 19, 2026. Title: Novel quantitative analysis method for biomolecular interactions. Applicant: Kyoto University. Application IB. The sequence listing filed with the application follows.

SEQUENCE LISTING (12 sequences)

SEQ ID NO: 1 - DNA, 16 bp, synthetic construct
  misc_feature 1..16: note = complementary sequence
  source 1..16: mol_type = other DNA
gcaatcaatcaacaac

SEQ ID NO: 2 - DNA, 16 bp, synthetic construct
  misc_feature 1..16: note = complementary sequence
  source 1..16: mol_type = other DNA
cttctacttacaccac

SEQ ID NO: 3 - DNA, 16 bp, synthetic construct
  misc_feature 1..16: note = complementary sequence
  source 1..16: mol_type = other DNA
cttctccattttccag

SEQ ID NO: 4 - DNA, 16 bp, synthetic construct
  misc_feature 1..16: note = complementary sequence
  source 1..16: mol_type = other DNA
gtgcgttctatcttcc

SEQ ID NO: 5 - DNA, 16 bp, synthetic construct
  misc_feature 1..16: note = complementary sequence
  source 1..16: mol_type = other DNA
ggtgatgatggtttgg

SEQ ID NO: 6 - DNA, 16 bp, synthetic construct
  misc_feature 1..16: note = complementary sequence
  source 1..16: mol_type = other DNA
cacgtaacaagatccc

SEQ ID NO: 7 - DNA, 16 bp, synthetic construct
  misc_feature 1..16: note = complementary sequence
  source 1..16: mol_type = other DNA
gtgatttgaaagttgc

SEQ ID NO: 8 - DNA, 16 bp, synthetic construct
  misc_feature 1..16: note = complementary sequence
  source 1..16: mol_type = other DNA
taatatggacgggaaa

SEQ ID NO: 9 - DNA, 16 bp, synthetic construct
  misc_feature 1..16: note = complementary sequence
  source 1..16: mol_type = other DNA
ttttctactcttcacg

SEQ ID NO: 10 - protein, 11 aa, synthetic construct
  REGION 1..11: note = complementary sequence
LPETGHHHHHH

SEQ ID NO: 11 - protein, 13 aa, synthetic construct
KFEKEKMNCKWMT

SEQ ID NO: 12 - protein, 13 aa, synthetic construct
KAEKEKMNCKAMT